European Patent Application EP 4 137 819 A1, published February 22, 2023. Title: NRF2 SCREENING ASSAYS AND RELATED METHODS AND COMPOSITIONS. Applicant: Biogen MA Inc. The sequence listing filed with the application follows.

SEQUENCE LISTING (18 sequences)

SEQ ID NO: 1-4 - skipped (4 entries)

SEQ ID NO: 5 - DNA, 24 bp, synthetic construct
  misc_feature 1..24: note = source = /="Description of Artificial Sequence: Syntheticconstruct"
  source 1..24: mol_type = other DNA
agtcacagtgagtcggcaaaattt

SEQ ID NO: 6 - DNA, 24 bp, synthetic construct
  misc_feature 1..24: note = source = /="Description of Artificial Sequence: Syntheticconstruct"
  source 1..24: mol_type = other DNA
agtcacagtgacttggcaaaatct

SEQ ID NO: 7 - DNA, 24 bp, synthetic construct
  misc_feature 1..24: note = source = /="Description of Artificial Sequence: Syntheticconstruct"
  source 1..24: mol_type = other DNA
agtcacagtgactcagcagaatct

SEQ ID NO: 8 - DNA, 24 bp, synthetic construct
  misc_feature 1..24: note = source = /="Description of Artificial Sequence: Syntheticconstruct"
  source 1..24: mol_type = other DNA
gctaatggtgacaaagcaactttc

SEQ ID NO: 9 - DNA, 24 bp, synthetic construct
  misc_feature 1..24: note = source = /="Description of Artificial Sequence: Syntheticconstruct"
  source 1..24: mol_type = other DNA
gctaatggtgacaaagcaactttc

SEQ ID NO: 10 - DNA, 24 bp, synthetic construct
  misc_feature 1..24: note = source = /="Description of Artificial Sequence: Syntheticconstruct"
  source 1..24: mol_type = other DNA
ctcaggcatgacattgcatttttc

SEQ ID NO: 11 - DNA, 24 bp, synthetic construct
  misc_feature 1..24: note = source = /="Description of Artificial Sequence: Syntheticconstruct"
  source 1..24: mol_type = other DNA
agtcactatgattcagcaacaaaa

SEQ ID NO: 12 - DNA, 24 bp, synthetic construct
  misc_feature 1..24: note = source = /="Description of Artificial Sequence: Syntheticconstruct"
  source 1..24: mol_type = other DNA
cctccccgtgactcagcgctttgt

SEQ ID NO: 13 - DNA, 24 bp, synthetic construct
  misc_feature 1..24: note = source = /="Description of Artificial Sequence: Syntheticconstruct"
  source 1..24: mol_type = other DNA
gaagacaatgactaagcagaaatc

SEQ ID NO: 14 - DNA, 24 bp, synthetic construct
  misc_feature 1..24: note = source = /="Description of Artificial Sequence: Syntheticconstruct"
  source 1..24: mol_type = other DNA
cccaaccatgacacagcataaaag

SEQ ID NO: 15 - skipped

SEQ ID NO: 16 - DNA, 20 bp, synthetic construct
  modified_base 11..13: mod_base = OTHER; note = a, c, g, t, unknown or other
  modified_base 4..5: mod_base = OTHER; note = a, c, g, t, unknown or other
  misc_feature 1..20: note = source = /="Description of Artificial Sequence: Syntheticconstruct"
  source 1..20: mol_type = other DNA
taannatgacnnngcaaaaa

SEQ ID NO: 17 - RNA, 21 nt, synthetic construct
  misc_feature 1..21: note = source = /="Description of Artificial Sequence: Syntheticoligonucleotide"
  source 1..21: mol_type = other RNA
tcattgaactgctctttggtt

SEQ ID NO: 18 - RNA, 21 nt, synthetic construct
  misc_feature 1..21: note = source = /="Description of Artificial Sequence: Syntheticoligonucleotide"
  source 1..21: mol_type = other RNA
gaattaaggcggtttgtcctt